European Patent Specification EP 2 984 170 B1, published May 20, 2026. Title: Antibody-Urease Conjugates. Applicant: Helix Biopharma Corp. The sequence listing filed with the application follows.

SEQUENCE LISTING (1 sequence)

SEQ ID NO: 1 - protein, 840 aa, Unknown
  Jack bean urease
MKLSPREVEKLGLHNAGYLAQKRLARGVRLNYTEAVALIASQIMEYARDGEKTVAQLMCLGQHLLGRRQVLPAVPHLLNAVQVEATFPDGTKLVTVHDPISRENGELQEALFGSLLPVPSLDKFAETKEDNRIPGEILCEDECLTLNIGRKAVILKVTSKGDRPIQVGSHYHFIEVNPYLTFDRRKAYGMRLNIAAGTAVRFEPGDCKSVTLVSIEGNKVIRGGNAIADGPVNETNLEAAMHAVRSKGFGHEEEKDASEGFTKEDPNCPFNTFIHRKEYANKYGPTTGDKIRLGDTNLLAEIEKDYALYGDECVFGGGKVIRDGMGQSCGHPPAISLDTVITNAVIIDYTGIIKADIGIKDGLIASIGKAGNPDIMNGVFSNMIIGANTEVIAGEGLIVTAGAIDCHVHYICPQLVYEAISSGITTLVGGGTGPAAGTRATTCTPSPTQMRLMLQSTDDLPLNFGFTGKGSSSKPDELHEIIKAGAMGLKLHEDWGSTPAAIDNCLTIAEHHDIQINIHTDTLNEAGFVEHSIAAFKGRTIHTYHSEGAGGGHAPDIIKVCGIKNVLPSSTNPTRPLTSNTIDEHLDMLMVCHHLDREIPEDLAFAHSRIRKKTIAAEDVLNDIGAISIISSDSQAMGRVGEVISRTWQTADKMKAQTGPLKCDSSDNDNFRIRRYIAKYTINPAIANGFSQYVGSVEVGKLADLVMWKPSFFGTKPEMVIKGGMVAWADIGDPNASIPTPEPVKMRPMYGTLGKAGGALSIAFVSKAALDQRVNVLYGLNKRVEAVSNVRKLTKLDMKLNDALPEITVDPESYTVKADGKLLCVSEATTVPLSRNYFLF